European Patent Specification EP 3 850 106 B1, published May 29, 2024. Title: METHODS OF IDENTIFYING DHA CANOLA NS-B50027-4. Applicant: NUSEED PTY LTD. The sequence listing filed with the application follows.

SEQUENCE LISTING (27 sequences)

SEQ ID NO: 1 - DNA, 15 bp, Artificial Sequence
  B. napus fragment of A02 replaced by transgenic insert
gtagcacgacaagtt

SEQ ID NO: 2 - DNA, 20 bp, Artificial Sequence
  B. napus fragment of A05 replaced by transgenic insert
cacggtggaggtcaccatgt

SEQ ID NO: 3 - DNA, 24 bp, Artificial Sequence
  Forward primer for junction of T-DNA insert on chromosome A05 (A05-286F)
gaacaacaaggaacagagcaacgt

SEQ ID NO: 4 - DNA, 24 bp, Artificial Sequence
  Reverse primer for junction of T-DNA insert on on chromosome A05 (A05-286R)
gacaatctgctagtggatctccca

SEQ ID NO: 5 - DNA, 20 bp, Artificial Sequence
  Forward primer for junction of T-DNA insert on on chromosome A02 (A05-282F)
cagatcttccaaggcctcgt

SEQ ID NO: 6 - DNA, 23 bp, Artificial Sequence
  Reverse primer for junction of T-DNA insert on chromosome A02 (A05-282R)
cgctcttatactgcactggttag

SEQ ID NO: 7 - DNA, 22 bp, Artificial Sequence
  Forward primer for internal reference gene HMG (hmg99F; control)
ggtcgtcctcctaaggcgaaag

SEQ ID NO: 8 - DNA, 20 bp, Artificial Sequence
  Reverse primer for internal reference gene HMG (hmg99R; control)
cttcttcggcggtcgtccac

SEQ ID NO: 9 - DNA, 189 bp, Artificial Sequence
  A02 genomic/transgene junction sequence used to design primers
ctccgccgccaacaaggcttgtagttaataggaatcattcagggattgtgattccgggcagtagtaattaataatatagtattagtatacagaacctcttatttagctaaaagattatgttcttaatgttgataagaagtttgagaaacaaatataattgagcttctgattagttgatcgtaattggtc

SEQ ID NO: 10 - DNA, 226 bp, Artificial Sequence
  A05 genomic/transgene junction sequence used to design primers
ttttcgtcgagttgctgaaactggacccaagccagtgtacggcgcaggaggtactttaagcttataaccctttgtctatcctttggctagcggctaatgttgatgaacttttttattcaaccgttggctaaggtaacactgatagtttaaactgaaggcgggaaacgacaatctgctagtggatctcccagtcacgacgttgtaaaacgggcgccccgcggaaagc

SEQ ID NO: 11 - DNA, 24 bp, Artificial Sequence
  Reference probe sequence for quantitative detection (hmg-P)
cggagccactcggtgccgcaactt

SEQ ID NO: 12 - DNA, 20 bp, Artificial Sequence
  Forward primer for A05up2 assay (A05up2F)
tctatcctttggctagcggc

SEQ ID NO: 13 - DNA, 21 bp, Artificial Sequence
  Reverse primer for A05up2 assay (A05up2R)
tgactgggagatccactagca

SEQ ID NO: 14 - DNA, 25 bp, Artificial Sequence
  Probe sequence for A05up2 assay (A05up2P)
caaccgttggctaaggtaacactga

SEQ ID NO: 15 - DNA, 26 bp, Artificial Sequence
  Forward primer for A02dn2 assay (A02dn2F)
acaaggcttgtagttaataggaatca

SEQ ID NO: 16 - DNA, 26 bp, Artificial Sequence
  Reverse primer for A02dn2 assay (A02dn2R)
acgatcaactaatcagaagctcaatt

SEQ ID NO: 17 - DNA, 22 bp, Artificial Sequence
  Probe sequence for A02dn2 assay (A02dn2P)
tcagggattgtgattccgggca

SEQ ID NO: 18 - DNA, 20 bp, Artificial Sequence
  Forward primer for junction between T-DNA and genomic DNA on Chromosome A05 (A05-200F)
tgttgtggtggtgacgattt

SEQ ID NO: 19 - DNA, 21 bp, Artificial Sequence
  Reverse primer for junction between T-DNA and genomic DNA on Chromosome A05 (A05-200R)
tccactagcagattgtcgttt

SEQ ID NO: 20 - DNA, 21 bp, Artificial Sequence
  Forward primer for junction between T-DNA and genomic DNA on Chromosome A02 (A02-258F)
cattgagcagtgaacaccaag

SEQ ID NO: 21 - DNA, 27 bp, Artificial Sequence
  Reverse primer for junction between T-DNA and genomic DNA on Chromosome A02 (A02-258R)
cagtttaaactatcagtgtttgaacac

SEQ ID NO: 22 - DNA, 18 bp, Artificial Sequence
  Forward primer for internal reference gene HMG as control (Hmg206F)
tccttccgtttcctcgcc

SEQ ID NO: 23 - DNA, 18 bp, Artificial Sequence
  Reverse primer for internal reference gene HMG as control (Hmg206R)
ttccacgccctctccgct

SEQ ID NO: 24 - DNA, 320 bp, Artificial Sequence
  Transgene junction region of NS-B50027-4 chromosome A02 for assay A02-282
ctgattctgcccgttcgactcagatcttccaaggcctcgtctccgagtccgctgcttctcgccgcgccgatcacttctccgccgccaacaaggcttgtagttaataggaatcattcagggattgtgattccgggcagtagtaattaataatatagtattagtatacagaacctcttatttagctaaaagattatgttcttaatgttgataagaagtttgagaaacaaatataattgagcttctgattagttgatcgtaattggtcattaataattgtatctaaccagtgcagtataagagcgtataagagcatcttcaaa

SEQ ID NO: 25 - DNA, 380 bp, Artificial Sequence
  Transgene junction region of NS-B50027-4 chromosome A05 for assay A05-286
tttctttacccaaatctagttcttgagaggatgaagcatcaccgaacagttctgcaactatccctcaaaagctttaaaatgaacaacaaggaacagagcaacgttccaaagatcccaaacgaaacatattatctatactaatactatattattaattactactgcccggaatcacaatccctgaatgattcctattaactacaagccttgttggcggcggagaagtgatcggcgcggcgagaagcagcggactcggagacgaggccttggaagatctgagtcgaacgggcggtaccgcgggcccgttttacaacgtcgtgactgggagatccactagcagattgtcgtttcccgccttcagtttaaactatcagtgtttg

SEQ ID NO: 26 - DNA, 480 bp, Artificial Sequence
  Transgene junction region of NS-B50027-4 chromosome A02 for assay A02-258
ctacgatggtactcaatgcggctaaggattgatgaagatggagatgttgcagatgagttcttggaagatgataactgtaagactttgcccagaaaatgcaaaacaaaagctgcaaaagtgagaggtttagtgatatcttctgatgggaaacttcagccattaatgcattgagcagtgaacaccaaggataaatatttactgattagtgtgtgattgaatcaaagaaaggttagaatctggttttcatttagccattcaatctcgatgtaaaatcggttagattctggttgttgatacttgagaacttgaaatgttttgtaactgtgaattttgttttgaaaatagacaagtgaatctgtttggggttgtgtgaaaacgtgtgagcaattgttggaggtgttcaaacactgatagtttaaactgaaggcgggaaacgacaatctgctagtggatctcccagtcacgacgttgtaaaacggg

SEQ ID NO: 27 - DNA, 640 bp, Artificial Sequence
  Transgene junction region of NS-B50027-4 chromosome A05 for assay A05-200
taatcatggaggagaagaaggatttttataaccatgtctctgttgcttgctgcttaaaccctatataattggaaactttttgttttagtctgtgtctgaaagtttctatattcgtattgtctattttgtaaagactaaaacaaaaatgcctatttttagtttgttcttgttccgcaacaccgttactgaactcttcgttcacttaaacagtttgtgtgtgtgagaaacagcgtaatgagctgctttggttgttgtggtggtgacgattttcgtcgagttgctgaaactggacccaagccagtgtacggcgcaggaggtactttaagcttataaccctttgtctatcctttggctagcggctaatgttgatgaacttttttattcaaccgttggctaaggtaacactgatagtttaaactgaaggcgggaaacgacaatctgctagtggatctcccagtcacgacgttgtaaaacgggcgccccgcggaaagcttgcggccgcggtaccgcccgttcgactcagatcttccaaggcctcgtctccgagtccgctgcttctcgccgcgccgatcacttctccgccgccaacaaggcttgtagttaataggaatcattcagggattgtgattccgggcagtag